European Patent Application EP 4 524 149 A1, published March 19, 2025. Title: USE OF ANTIGENIC SHORT PEPTIDE IN SCREENING DRUG FOR TREATING HPV-RELATED DISEASES AND TCR SCREENED BY SAME. Applicant: Guangzhou Medical University. Application WO. The sequence listing filed with the application follows.

SEQUENCE LISTING (46 sequences)

SEQ ID NO: 1 - protein, 9 aa, synthetic construct
TTLEQQYNK

SEQ ID NO: 2 - protein, 10 aa, synthetic construct
GTTLEQQYNK

SEQ ID NO: 3 - protein, 6 aa, synthetic construct
SSYSPS

SEQ ID NO: 4 - protein, 8 aa, synthetic construct
YTSAATLV

SEQ ID NO: 5 - protein, 12 aa, synthetic construct
VVSLSGGYNKLI

SEQ ID NO: 6 - protein, 5 aa, synthetic construct
SGDLS

SEQ ID NO: 7 - protein, 6 aa, synthetic construct
YYNGEE

SEQ ID NO: 8 - protein, 10 aa, synthetic construct
ASSVTGSGYT

SEQ ID NO: 9 - protein, 5 aa, synthetic construct
TTLSN

SEQ ID NO: 10 - protein, 7 aa, synthetic construct
LVKSGEV

SEQ ID NO: 11 - protein, 13 aa, synthetic construct
AGPKITGGGNKLT

SEQ ID NO: 12 - protein, 13 aa, synthetic construct
ASSVGGGPNYGYT

SEQ ID NO: 13 - protein, 13 aa, synthetic construct
AGPILTGGGNKLT

SEQ ID NO: 14 - protein, 13 aa, synthetic construct
ASGLSGPNTGELF

SEQ ID NO: 15 - protein, 13 aa, synthetic construct
AGPVLTGGGNKLT

SEQ ID NO: 16 - protein, 13 aa, synthetic construct
ASSVGGPNTGELF

SEQ ID NO: 17 - protein, 19 aa, synthetic construct
MLLLLVPVLEVIFTLGGTR

SEQ ID NO: 18 - protein, 19 aa, synthetic construct
MGFRLLCCVAFCLLGAGPV

SEQ ID NO: 19 - protein, 18 aa, synthetic construct
MLLITSMLVLWMQLSQVN

SEQ ID NO: 20 - protein, 134 aa, synthetic construct
MLLLLVPVLEVIFTLGGTRAQSVTQLDSHVSVSEGTPVLLRCNYSSSYSPSLFWYVQHPNKGLQLLLKYTSAATLVKGINGFEAEFKKSETSFHLTKPSAHMSDAAEYFCVVSLSGGYNKLIFGAGTRLAVHPY

SEQ ID NO: 21 - protein, 130 aa, synthetic construct
MGFRLLCCVAFCLLGAGPVDSGVTQTPKHLITATGQRVTLRCSPRSGDLSVYWYQQSLDQGLQFLIQYYNGEERAKGNILERFSAQQFPDLHSELNLSSLELGDSALYFCASSVTGSGYTFGSGTRLTVV

SEQ ID NO: 22 - protein, 132 aa, synthetic construct
MLLITSMLVLWMQLSQVNGQQVMQIPQYQHVQEGEDFTTYCNSSTTLSNIQWYKQRPGGHPVFLIQLVKSGEVKKQKRLTFQFGEAKKNSSLHITATQTTDVGTYFCAGPKITGGGNKLTFGTGTQLKVELN

SEQ ID NO: 23 - protein, 133 aa, synthetic construct
MGFRLLCCVAFCLLGAGPVDSGVTQTPKHLITATGQRVTLRCSPRSGDLSVYWYQQSLDQGLQFLIQYYNGEERAKGNILERFSAQQFPDLHSELNLSSLELGDSALYFCASSVGGGPNYGYTFGSGTRLTVV

SEQ ID NO: 24 - protein, 132 aa, synthetic construct
MLLITSMLVLWMQLSQVNGQQVMQIPQYQHVQEGEDFTTYCNSSTTLSNIQWYKQRPGGHPVFLIQLVKSGEVKKQKRLTFQFGEAKKNSSLHITATQTTDVGTYFCAGPILTGGGNKLTFGTGTQLKVELN

SEQ ID NO: 25 - protein, 133 aa, synthetic construct
MGFRLLCCVAFCLLGAGPVDSGVTQTPKHLITATGQRVTLRCSPRSGDLSVYWYQQSLDQGLQFLIQYYNGEERAKGNILERFSAQQFPDLHSELNLSSLELGDSALYFCASGLSGPNTGELFFGEGSRLTVL

SEQ ID NO: 26 - protein, 132 aa, synthetic construct
MLLITSMLVLWMQLSQVNGQQVMQIPQYQHVQEGEDFTTYCNSSTTLSNIQWYKQRPGGHPVFLIQLVKSGEVKKQKRLTFQFGEAKKNSSLHITATQLTDVGTYFCAGPVLTGGGNKLTFGTGTQLKVELN

SEQ ID NO: 27 - protein, 133 aa, synthetic construct
MGFRLLCCVAFCLLGAGPVDSGVTQTPRYLITATGQRVTLRCSPRSGDLSVYWYQQSLDQGLQFLIQYYNGEERAKGNILERFSAQQFPDLHSELNLSSLELGDSALYFCASSVGGPNTGELFFGEGSRLTVL

SEQ ID NO: 28 - protein, 136 aa, synthetic construct
IQNPEPAVYQLKDPRSQDSTLCLFTDFDSQINVPKTMESGTFITDKCVLDMKAMDSKSNGAIAWSNQTSFTCQDIFKETNATYPSSDVPCDATLTEKSFETDMNLNFQNLSVMGLRILLLKVAGFNLLMTLRLWSS

SEQ ID NO: 29 - protein, 173 aa, synthetic construct
EDLRNVTPPKVSLFEPSKAEIANKQKATLVCLARGFFPDHVELSWWVNGKEVHSGVCTDPQAYKESNYSYCLSSRLRVSATFWHNPRNHFRCQVQFHGLSEEDKWPEGSPKPVTQNISAEAWGRADCGITSASYHQGVLSATILYEILLGKATLYAVLVSGLVLMAMVKKKNS

SEQ ID NO: 30 - DNA, 810 bp, synthetic construct
  source 1..810: mol_type = other DNA
atgctcctgctgctcgtcccagtgctcgaggtgatttttactctgggaggaaccagagcccagtcggtgacccagcttgacagccacgtctctgtctctgaaggaaccccggtgctgctgaggtgcaactactcatcttcttattcaccatctctcttctggtatgtgcaacaccccaacaaaggactccagcttctcctgaagtacacatcagcggccaccctggttaaaggcatcaacggttttgaggctgaatttaagaagagtgaaacctccttccacctgacgaaaccctcagcccatatgagcgacgcggctgagtacttctgtgttgtgagtctttctggtggctacaataagctgatttttggagcagggaccaggctggctgtacacccatatatccagaatccagagcccgccgtgtatcagctgaaggacccaaggagccaggattccaccctgtgcctgttcacagactttgatagccagatcaacgtgcccaagaccatggagtccggcaccttcatcacagacaagtgcgtgctggatatgaaggccatggactctaagagcaacggcgccatcgcctggagcaatcagacctccttcacatgccaggatatctttaaggagaccaatgccacatatccttcctctgacgtgccatgtgatgccaccctgacagagaagtccttcgagaccgacatgaacctgaattttcagaacctgtctgtgatgggcctgcgcatcctgctgctgaaggtggccggcttcaatctgctgatgaccctgaggctgtggagctcc

SEQ ID NO: 31 - DNA, 909 bp, synthetic construct
  source 1..909: mol_type = other DNA
atgggcttcaggctcctctgctgtgtggccttttgtctcctgggagcaggcccagtggattctggagtcacacaaaccccaaagcacctgatcacagcaactggacagcgagtgacgctgagatgctcccctaggtctggagacctctctgtgtactggtaccaacagagcctggaccagggcctccagttcctcattcagtattataatggagaagagagagcaaaaggaaacattcttgaacgattctccgcacaacagttccctgacttgcactctgaactaaacctgagctctctggagctgggggactcagctttgtatttctgtgccagcagcgtgacagggagtggctacaccttcggttcggggaccaggttaaccgttgtagaggatctgaggaacgtgacaccccctaaggtgtctctgttcgagcccagcaaggccgagatcgccaataagcagaaggccaccctggtgtgcctggcaaggggcttctttcctgatcacgtggagctgtcttggtgggtgaacggcaaggaggtgcacagcggcgtgtgcaccgacccacaggcctacaaggagtccaattactcttattgtctgagctcccggctgagagtgtccgccacattttggcacaaccctagaaatcacttcaggtgccaggtgcagtttcacggcctgagcgaggaggataagtggccagagggatccccaaagcctgtgacccagaacatctctgccgaggcatggggaagggcagactgtggaatcacatccgcctcttatcaccagggcgtgctgagcgccaccatcctgtacgagatcctgctgggcaaggccacactgtatgccgtgctggtgagcggcctggtgctgatggccatggtgaagaagaagaactcc

SEQ ID NO: 32 - DNA, 804 bp, synthetic construct
  source 1..804: mol_type = other DNA
atgctactcatcacatcaatgttggtcttatggatgcaattgtcacaggtgaatggacaacaggtaatgcaaattcctcagtaccagcatgtacaagaaggagaggacttcaccacgtactgcaattcctcaactactttaagcaatatacagtggtataagcaaaggcctggtggacatcccgtttttttgatacagttagtgaagagtggagaagtgaagaagcagaaaagactgacatttcagtttggagaagcaaaaaagaacagctccctgcacatcacagccacccagactacagatgtaggaacctacttctgtgcagggccgaaaatcacgggaggaggaaacaaactcacctttgggacaggcactcagctaaaagtggaactcaatatccagaatccagagcccgccgtgtatcagctgaaggacccaaggagccaggattccaccctgtgcctgttcacagactttgatagccagatcaacgtgcccaagaccatggagtccggcaccttcatcacagacaagtgcgtgctggatatgaaggccatggactctaagagcaacggcgccatcgcctggagcaatcagacctccttcacatgccaggatatctttaaggagaccaatgccacatatccttcctctgacgtgccatgtgatgccaccctgacagagaagtccttcgagaccgacatgaacctgaattttcagaacctgtctgtgatgggcctgcgcatcctgctgctgaaggtggccggcttcaatctgctgatgaccctgaggctgtggagctcc

SEQ ID NO: 33 - DNA, 918 bp, synthetic construct
  source 1..918: mol_type = other DNA
atgggcttcaggctcctctgctgtgtggccttttgtctcctgggagcaggcccagtggattctggagtcacacaaaccccaaagcacctgatcacagcaactggacagcgagtgacgctgagatgctcccctaggtctggagacctctctgtgtactggtaccaacagagcctggaccagggcctccagttcctcattcagtattataatggagaagagagagcaaaaggaaacattcttgaacgattctccgcacaacagttccctgacttgcactctgaactaaacctgagctctctggagctgggggactcagctttgtatttctgtgccagcagcgtaggcgggggccctaactatggctacaccttcggttcggggaccaggttaaccgttgtagaggatctgaggaacgtgacaccccctaaggtgtctctgttcgagcccagcaaggccgagatcgccaataagcagaaggccaccctggtgtgcctggcaaggggcttctttcctgatcacgtggagctgtcttggtgggtgaacggcaaggaggtgcacagcggcgtgtgcaccgacccacaggcctacaaggagtccaattactcttattgtctgagctcccggctgagagtgtccgccacattttggcacaaccctagaaatcacttcaggtgccaggtgcagtttcacggcctgagcgaggaggataagtggccagagggatccccaaagcctgtgacccagaacatctctgccgaggcatggggaagggcagactgtggaatcacatccgcctcttatcaccagggcgtgctgagcgccaccatcctgtacgagatcctgctgggcaaggccacactgtatgccgtgctggtgagcggcctggtgctgatggccatggtgaagaagaagaactcc

SEQ ID NO: 34 - DNA, 804 bp, synthetic construct
  source 1..804: mol_type = other DNA
atgctactcatcacatcaatgttggtcttatggatgcaattgtcacaggtgaatggacaacaggtaatgcaaattcctcagtaccagcatgtacaagaaggagaggacttcaccacgtactgcaattcctcaactactttaagcaatatacagtggtataagcaaaggcctggtggacatcccgtttttttgatacagttagtgaagagtggagaagtgaagaagcagaaaagactgacatttcagtttggagaagcaaaaaagaacagctccctgcacatcacagccacccagactacagatgtaggaacctacttctgtgcaggccccatactcacgggaggaggaaacaaactcacctttgggacaggcactcagctaaaagtggaactcaatatccagaatccagagcccgccgtgtatcagctgaaggacccaaggagccaggattccaccctgtgcctgttcacagactttgatagccagatcaacgtgcccaagaccatggagtccggcaccttcatcacagacaagtgcgtgctggatatgaaggccatggactctaagagcaacggcgccatcgcctggagcaatcagacctccttcacatgccaggatatctttaaggagaccaatgccacatatccttcctctgacgtgccatgtgatgccaccctgacagagaagtccttcgagaccgacatgaacctgaattttcagaacctgtctgtgatgggcctgcgcatcctgctgctgaaggtggccggcttcaatctgctgatgaccctgaggctgtggagctcc

SEQ ID NO: 35 - DNA, 918 bp, synthetic construct
  source 1..918: mol_type = other DNA
atgggcttcaggctcctctgctgtgtggccttttgtctcctgggagcaggcccagtggattctggagtcacacaaaccccaaagcacctgatcacagcaactggacagcgagtgacgctgagatgctcccctaggtctggagacctctctgtgtactggtaccaacagagcctggaccagggcctccagttcctcattcagtattataatggagaagagagagcaaaaggaaacattcttgaacgattctccgcacaacagttccctgacttgcactctgaactaaacctgagctctctggagctgggggactcagctttgtatttctgtgccagcgggctttcaggaccgaacaccggggagctgttttttggagaaggctctaggctgaccgtactggaggatctgaggaacgtgacaccccctaaggtgtctctgttcgagcccagcaaggccgagatcgccaataagcagaaggccaccctggtgtgcctggcaaggggcttctttcctgatcacgtggagctgtcttggtgggtgaacggcaaggaggtgcacagcggcgtgtgcaccgacccacaggcctacaaggagtccaattactcttattgtctgagctcccggctgagagtgtccgccacattttggcacaaccctagaaatcacttcaggtgccaggtgcagtttcacggcctgagcgaggaggataagtggccagagggatccccaaagcctgtgacccagaacatctctgccgaggcatggggaagggcagactgtggaatcacatccgcctcttatcaccagggcgtgctgagcgccaccatcctgtacgagatcctgctgggcaaggccacactgtatgccgtgctggtgagcggcctggtgctgatggccatggtgaagaagaagaactcc

SEQ ID NO: 36 - DNA, 804 bp, synthetic construct
  source 1..804: mol_type = other DNA
atgctactcatcacatcaatgttggtcttatggatgcaattgtcacaggtgaatggacaacaggtaatgcaaattcctcagtaccagcatgtacaagaaggagaggacttcaccacgtactgcaattcctcaactactttaagcaatatacagtggtataagcaaaggcctggtggacatcccgtttttttgatacagttagtgaagagtggagaagtgaagaagcagaaaagactgacatttcagtttggagaagcaaaaaagaacagctccctgcacatcacagccacccagactacagatgtaggaacctacttctgtgcagggccggtactcacgggaggaggaaacaaactcacctttgggacaggcactcagctaaaagtggaactcaatatccagaatccagagcccgccgtgtatcagctgaaggacccaaggagccaggattccaccctgtgcctgttcacagactttgatagccagatcaacgtgcccaagaccatggagtccggcaccttcatcacagacaagtgcgtgctggatatgaaggccatggactctaagagcaacggcgccatcgcctggagcaatcagacctccttcacatgccaggatatctttaaggagaccaatgccacatatccttcctctgacgtgccatgtgatgccaccctgacagagaagtccttcgagaccgacatgaacctgaattttcagaacctgtctgtgatgggcctgcgcatcctgctgctgaaggtggccggcttcaatctgctgatgaccctgaggctgtggagctcc

SEQ ID NO: 37 - DNA, 918 bp, synthetic construct
  source 1..918: mol_type = other DNA
atgggcttcaggctcctctgctgtgtggccttttgtctcctgggagcaggcccagtggattctggagtcacacaaaccccaaagcacctgatcacagcaactggacagcgagtgacgctgagatgctcccctaggtctggagacctctctgtgtactggtaccaacagagcctggaccagggcctccagttcctcattcagtattataatggagaagagagagcaaaaggaaacattcttgaacgattctccgcacaacagttccctgacttgcactctgaactaaacctgagctctctggagctgggggactcagctttgtatttctgtgccagcagcgtggggggaccgaacaccggggagctgttttttggagaaggctctaggctgaccgtactggaggatctgaggaacgtgacaccccctaaggtgtctctgttcgagcccagcaaggccgagatcgccaataagcagaaggccaccctggtgtgcctggcaaggggcttctttcctgatcacgtggagctgtcttggtgggtgaacggcaaggaggtgcacagcggcgtgtgcaccgacccacaggcctacaaggagtccaattactcttattgtctgagctcccggctgagagtgtccgccacattttggcacaaccctagaaatcacttcaggtgccaggtgcagtttcacggcctgagcgaggaggataagtggccagagggatccccaaagcctgtgacccagaacatctctgccgaggcatggggaagggcagactgtggaatcacatccgcctcttatcaccagggcgtgctgagcgccaccatcctgtacgagatcctgctgggcaaggccacactgtatgccgtgctggtgagcggcctggtgctgatggccatggtgaagaagaagaactcc

SEQ ID NO: 38 - protein, 367 aa, synthetic construct
MAVMAPRTLLLLLSGALALTQTWAGSHSMRYFYTSVSRPGRGEPRFIAVGYVDDTQFVRFDSDAASQRMEPRAPWIEQEGPEYWDQETRNVKAQSQTDRVDLGTLRGYYNQSEDGSHTIQIMYGCDVGPDGRFLRGYRQDAYDGKDYIALNEDLRSWTAADMAAQITKRKWEAAHAAEQQRAYLEGRCVEWLRRYLENGKETLQRTDPPKTHMTHHPISDHEATLRCWALGFYPAEITLTWQRDGEDQTQDTELVETRPAGDGTFQKWAAVVVPSGEEQRYTCHVQHEGLPKPLTLRWELSSQPTIPIVGIIAGLVLLGAVITGAVVAAVMWRRKSSDRKGGSYTQAASSDSAQGSDVSLTACKVSR

SEQ ID NO: 39 - DNA, 402 bp, synthetic construct
  source 1..402: mol_type = other DNA
atgctcctgctgctcgtcccagtgctcgaggtgatttttactctgggaggaaccagagcccagtcggtgacccagcttgacagccacgtctctgtctctgaaggaaccccggtgctgctgaggtgcaactactcatcttcttattcaccatctctcttctggtatgtgcaacaccccaacaaaggactccagcttctcctgaagtacacatcagcggccaccctggttaaaggcatcaacggttttgaggctgaatttaagaagagtgaaacctccttccacctgacgaaaccctcagcccatatgagcgacgcggctgagtacttctgtgttgtgagtctttctggtggctacaataagctgatttttggagcagggaccaggctggctgtacacccatat

SEQ ID NO: 40 - DNA, 390 bp, synthetic construct
  source 1..390: mol_type = other DNA
atgggcttcaggctcctctgctgtgtggccttttgtctcctgggagcaggcccagtggattctggagtcacacaaaccccaaagcacctgatcacagcaactggacagcgagtgacgctgagatgctcccctaggtctggagacctctctgtgtactggtaccaacagagcctggaccagggcctccagttcctcattcagtattataatggagaagagagagcaaaaggaaacattcttgaacgattctccgcacaacagttccctgacttgcactctgaactaaacctgagctctctggagctgggggactcagctttgtatttctgtgccagcagcgtgacagggagtggctacaccttcggttcggggaccaggttaaccgttgta

SEQ ID NO: 41 - DNA, 396 bp, synthetic construct
  source 1..396: mol_type = other DNA
atgctactcatcacatcaatgttggtcttatggatgcaattgtcacaggtgaatggacaacaggtaatgcaaattcctcagtaccagcatgtacaagaaggagaggacttcaccacgtactgcaattcctcaactactttaagcaatatacagtggtataagcaaaggcctggtggacatcccgtttttttgatacagttagtgaagagtggagaagtgaagaagcagaaaagactgacatttcagtttggagaagcaaaaaagaacagctccctgcacatcacagccacccagactacagatgtaggaacctacttctgtgcagggccgaaaatcacgggaggaggaaacaaactcacctttgggacaggcactcagctaaaagtggaactcaat

SEQ ID NO: 42 - DNA, 399 bp, synthetic construct
  source 1..399: mol_type = other DNA
atgggcttcaggctcctctgctgtgtggccttttgtctcctgggagcaggcccagtggattctggagtcacacaaaccccaaagcacctgatcacagcaactggacagcgagtgacgctgagatgctcccctaggtctggagacctctctgtgtactggtaccaacagagcctggaccagggcctccagttcctcattcagtattataatggagaagagagagcaaaaggaaacattcttgaacgattctccgcacaacagttccctgacttgcactctgaactaaacctgagctctctggagctgggggactcagctttgtatttctgtgccagcagcgtaggcgggggccctaactatggctacaccttcggttcggggaccaggttaaccgttgta

SEQ ID NO: 43 - DNA, 396 bp, synthetic construct
  source 1..396: mol_type = other DNA
atgctactcatcacatcaatgttggtcttatggatgcaattgtcacaggtgaatggacaacaggtaatgcaaattcctcagtaccagcatgtacaagaaggagaggacttcaccacgtactgcaattcctcaactactttaagcaatatacagtggtataagcaaaggcctggtggacatcccgtttttttgatacagttagtgaagagtggagaagtgaagaagcagaaaagactgacatttcagtttggagaagcaaaaaagaacagctccctgcacatcacagccacccagactacagatgtaggaacctacttctgtgcaggccccatactcacgggaggaggaaacaaactcacctttgggacaggcactcagctaaaagtggaactcaat

SEQ ID NO: 44 - DNA, 399 bp, synthetic construct
  source 1..399: mol_type = other DNA
atgggcttcaggctcctctgctgtgtggccttttgtctcctgggagcaggcccagtggattctggagtcacacaaaccccaaagcacctgatcacagcaactggacagcgagtgacgctgagatgctcccctaggtctggagacctctctgtgtactggtaccaacagagcctggaccagggcctccagttcctcattcagtattataatggagaagagagagcaaaaggaaacattcttgaacgattctccgcacaacagttccctgacttgcactctgaactaaacctgagctctctggagctgggggactcagctttgtatttctgtgccagcgggctttcaggaccgaacaccggggagctgttttttggagaaggctctaggctgaccgtactg

SEQ ID NO: 45 - DNA, 396 bp, synthetic construct
  source 1..396: mol_type = other DNA
atgctactcatcacatcaatgttggtcttatggatgcaattgtcacaggtgaatggacaacaggtaatgcaaattcctcagtaccagcatgtacaagaaggagaggacttcaccacgtactgcaattcctcaactactttaagcaatatacagtggtataagcaaaggcctggtggacatcccgtttttttgatacagttagtgaagagtggagaagtgaagaagcagaaaagactgacatttcagtttggagaagcaaaaaagaacagctccctgcacatcacagccacccagactacagatgtaggaacctacttctgtgcagggccggtactcacgggaggaggaaacaaactcacctttgggacaggcactcagctaaaagtggaactcaat

SEQ ID NO: 46 - DNA, 399 bp, synthetic construct
  source 1..399: mol_type = other DNA
atgggcttcaggctcctctgctgtgtggccttttgtctcctgggagcaggcccagtggattctggagtcacacaaaccccaaagcacctgatcacagcaactggacagcgagtgacgctgagatgctcccctaggtctggagacctctctgtgtactggtaccaacagagcctggaccagggcctccagttcctcattcagtattataatggagaagagagagcaaaaggaaacattcttgaacgattctccgcacaacagttccctgacttgcactctgaactaaacctgagctctctggagctgggggactcagctttgtatttctgtgccagcagcgtggggggaccgaacaccggggagctgttttttggagaaggctctaggctgaccgtactg